European Patent Application EP 4 324 526 A2, published February 21, 2024. Title: IMMUNOGENIC ANTI-INFLAMMATORY COMPOSITIONS. Applicant: QU BIOLOGICS INC. Application EP. The sequence listing filed with the application follows.

SEQUENCE LISTING (4 sequences)

SEQ ID NO: 1 - DNA, 19 bp, synthetic construct
  misc_feature 1..19: note = primer
  source 1..19: mol_type = other DNA
cgctttgccacggacgaga

SEQ ID NO: 2 - DNA, 19 bp, synthetic construct
  misc_feature 1..19: note = primer
  source 1..19: mol_type = other DNA
aggaaggcagcgggcacat

SEQ ID NO: 3 - DNA, 20 bp, synthetic construct
  misc_feature 1..20: note = primer
  source 1..20: mol_type = other DNA
ggtccaccctgacctatgtg

SEQ ID NO: 4 - DNA, 20 bp, synthetic construct
  misc_feature 1..20: note = primer
  source 1..20: mol_type = other DNA
gcaagccaatgtacacgatg